European Patent Application EP 4 684 805 A1, published January 28, 2026. Title: Selective Antibody-Drug Conjugates for Targeted Cancer Therapy. Applicant: Universitätsmedizin der Johannes Gutenberg-Universität Mainz. The sequence listing filed with the application follows.

SEQUENCE LISTING (9 sequences)

SEQ ID NO: 1 - protein, 8 aa, Mus musculus
GFTFSDYW

SEQ ID NO: 2 - protein, 10 aa, Mus musculus
IRLKSNNYAA

SEQ ID NO: 3 - protein, 8 aa, Mus musculus
TFGNSFAY

SEQ ID NO: 4 - protein, 9 aa, Mus musculus
TGAVTTNNY

SEQ ID NO: 5 - skipped

SEQ ID NO: 6 - protein, 9 aa, Mus musculus
ALWYSNHWV

SEQ ID NO: 7 - protein, 117 aa, Mus musculus
EVKLEESGGGLVQPGGSMKLSCVASGFTFSDYWMNWVRQSPEKGLEWVADIRLKSNNYAAHYAESVKGRFTVSRDDSKSSVYLQMNNLRTEDTGFYYCTFGNSFAYWGQGTLVTVSA

SEQ ID NO: 8 - protein, 109 aa, Mus musculus
QAVVTQESALTTSPGETVTLTCRSSTGAVTTNNYANWVQEKPDHLFTGLIGGTNNRGPGVPARFSGSLIGDKAALTITGAQTEDEAIYFCALWYSNHWVFGGGTKLTVL

SEQ ID NO: 9 - protein, 246 aa, Mus musculus
EVKLEESGGGLVQPGGSMKLSCVASGFTFSDYWMNWVRQSPEKGLEWVADIRLKSNNYAAHYAESVKGRFTVSRDDSKSSVYLQMNNLRTEDTGFYYCTFGNSFAYWGQGTLVTVSAGGGGSGGGGSGGGGSGGGGSQAVVTQESALTTSPGETVTLTCRSSTGAVTTNNYANWVQEKPDHLFTGLIGGTNNRGPGVPARFSGSLIGDKAALTITGAQTEDEAIYFCALWYSNHWVFGGGTKLTVL